European Patent Specification EP 3 508 210 B1, published March 20, 2024. Title: A composition for treating atopic dermatitis comprising the extract of herbal mixture. Applicant: University-Industry Cooperation Group of Kyung Hee University. The sequence listing filed with the application follows.

SEQUENCE LISTING (20 sequences)

SEQ ID NO: 1 - DNA, 20 bp, Artificial Sequence
  IL-4 forward primer
tcggcattttgaacgaggtc

SEQ ID NO: 2 - DNA, 20 bp, Artificial Sequence
  IL-4 reverse primer
gaaaagcccgaaagagtctc

SEQ ID NO: 3 - DNA, 22 bp, Artificial Sequence
  IL-6 forward primer
caagagacttccatccagttgc

SEQ ID NO: 4 - DNA, 21 bp, Artificial Sequence
  IL-6 reverse primer
ttgccgagttctcaaagtgac

SEQ ID NO: 5 - DNA, 20 bp, Artificial Sequence
  COX-2 forward primer
aagacttgccaggctgaact

SEQ ID NO: 6 - DNA, 21 bp, Artificial Sequence
  COX-2 reverse primer
cttctgcagtcccaggttcaa

SEQ ID NO: 7 - DNA, 27 bp, Artificial Sequence
  iNOS forward primer
aatggcaacatcaggtcggccatcact

SEQ ID NO: 8 - DNA, 27 bp, Artificial Sequence
  iNOS reverse primer
gctgtgtgtcacagaagtctcgaactc

SEQ ID NO: 9 - DNA, 21 bp, Artificial Sequence
  TNF-a forward primer
atgagcacagaaagcatgatc

SEQ ID NO: 10 - DNA, 21 bp, Artificial Sequence
  TNF-a reverse primer
tacaggcttgtcactggaatt

SEQ ID NO: 11 - DNA, 21 bp, Artificial Sequence
  GAPDH forward primer
gaggggccatccacagtcttc

SEQ ID NO: 12 - DNA, 21 bp, Artificial Sequence
  GAPDH reverse primer
catcaccatcttccaggagcg

SEQ ID NO: 13 - DNA, 20 bp, Artificial Sequence
  IL-4 forward primer
tgcctccaagaacacaactg

SEQ ID NO: 14 - DNA, 20 bp, Artificial Sequence
  IL-4 reverse primer
ctctggttggcttccttcac

SEQ ID NO: 15 - DNA, 21 bp, Artificial Sequence
  IL-6 forward primer
aaccttccaaagatggctagg

SEQ ID NO: 16 - DNA, 21 bp, Artificial Sequence
  IL-6 reverse primer
caggaactggatcaggacttt

SEQ ID NO: 17 - DNA, 20 bp, Artificial Sequence
  IL-13 forward primer
ggtcaacatcacccagaacc

SEQ ID NO: 18 - DNA, 20 bp, Artificial Sequence
  IL-13 reverse primer
tttacaaactgggccacctc

SEQ ID NO: 19 - DNA, 20 bp, Artificial Sequence
  GAPDH forward primer
cgtcttcaccaccatggaga

SEQ ID NO: 20 - DNA, 20 bp, Artificial Sequence
  GAPDH reverse primer
cggccatcacgccacagttt